European Patent Specification EP 3 823 979 B1, published December 18, 2024. Title: METHODS FOR SCREENING AND IDENTIFYING AGENTS THAT INHIBIT OR MODULATE THE NUCLEAR EGRESS COMPLEX OF HERPESVIRUSES. Applicant: AiCuris GmbH & Co. KG. The sequence listing filed with the application follows.

SEQUENCE LISTING (62 sequences)

SEQ ID NO: 1 - protein, 413 aa, Artificial Sequence
  Fusion protein of HCMV-NEC proteins pUL50 protein consisting of pUL50 (1-171) is fused via a GGSGSGGS linker to pUL53 (59-292).
MEMNKVLHQDLVQATRRILKLGPSELRVTDAGLICKNPNYSVCDAMLKTDTVYCVEYLLSYWESRTDHVPCFIFKNTGCAVSLCCFVRAPVKLVSPARHVGEFNVLKVNESLIVTLKDIEEIKPSAYGVLTKCVVRKSNSASVFNIELIAFGPENEGEYENLLRELYAKKAGGSGSGGSLTLHDLHDIFREHPELELKYLNMMKMAITGKESICLPFNFHSHRQHTCLDISPYGNEQVSRIACTSCEDNRILPTASDAMVAFINQTSNIMKNRNFYYGFCKSSELLKLSTNQPPIFQIYYLLHAANHDIVPFMHAEDGRLHMHVIFENPDVHIPCDCITQMLTAAREDYSVTLNIVRDHVVISVLCHAVSASSVKIDVTILQRKIDEMDIPNDVSESFERYKELIQELCQSSG

SEQ ID NO: 2 - protein, 208 aa, Artificial Sequence
  pUL50 protein consisting of pUL50 (1-171) is fused via a GGSGSGGS linker to pUL53 (59-87).
MEMNKVLHQDLVQATRRILKLGPSELRVTDAGLICKNPNYSVCDAMLKTDTVYCVEYLLSYWESRTDHVPCFIFKNTGCAVSLCCFVRAPVKLVSPARHVGEFNVLKVNESLIVTLKDIEEIKPSAYGVLTKCVVRKSNSASVFNIELIAFGPENEGEYENLLRELYAKKAGGSGSGGSLTLHDLHDIFREHPELELKYLNMMKMAIT

SEQ ID NO: 3 - protein, 438 aa, Human herpesvirus 8
MASPEERLLDELNNVIVSFLCDSGSLEVERCSGAHVFSRGSSQPLCTVKLRHGQIYHLEFVYKFLAFKLKNCNYPSSPVFVISNNGLATTLRCFLHEPSGLRSGQSGPCLGLSTDVDLPKNSIIMLGQDDFIKFKSPLVFPAELDLLKSMVVCRAYITEHRTTMQFLVFQAANAQKASRVMDMISDMSQQLSGGSGSDRSHFSLRDFFRGISANFELGKDFLREMNTPIHVSEAVFLPLSLCTLSPGRCLRLSPFGHSLTLGSHCEICINRSQVHVPQEFSSTQLSFFNNVHKIIPNKTFYVSLLSSSPSAVKAGLSQPSLLYAYLVTGHFCGTICPIFSTNGKGRLIMHLLLQGTSLHIPETCLKLLCENIGPTYELAVDLVGDAFCIKVSPRDTVYEKAVNVDEDAIYEAIKDLECGDELRLQIINYTQLILENKQ

SEQ ID NO: 4 - protein, 230 aa, Artificial Sequence
  EBV BFRF1 consisting of EBV BFRF1 (Uniprot entry: V5KTU9, 1- MASPEERLLD .. SDMSQQLS-192) is fused via a GGSGS linker to EBV BFLF2 (Uniprot entry: K9UT32, 78-DRSHFSLRD...... -110)
MASPEERLLDELNNVIVSFLCDSGSLEVERCSGAHVFSRGSSQPLCTVKLRHGQIYHLEFVYKFLAFKLKNCNYPSSPVFVISNNGLATTLRCFLHEPSGLRSGQSGPCLGLSTDVDLPKNSIIMLGQDDFIKFKSPLVFPAELDLLKSMVVCRAYITEHRTTMQFLVFQAANAQKASRVMDMISDMSQQLSGGSGSDRSHFSLRDFFRGISANFELGKDFLREMNTPIH

SEQ ID NO: 5 - protein, 439 aa, Artificial Sequence
  VZV orf24 consisting of VZV orf24 (Uniprot entry: Q6QCN1, 16- GDNLLQRI .. TDAYM-189) is fused via a GGSGSGGS linker to VZV orf27 (Uniprot entry: Q6QCM8, 77-SKERSV.... FDDFVPPR-333)
GDNLLQRIRLVVPSALQCCDGDLPIFDPQRPPARCVFQFNGEDNVSEAFPVEYIMRLMANWAQVDCDPYIKIQNTGVSVLFQGFFFRPTNAPVAEVSIDSNNVILSSTLSTGINLSALESIKRGGGIDRRPLQALMWVNCFVRMPYVQLSFRFMGPEDPSRTIKLMARATDAYMGGSGSGGSSKERSVYRHYFNYIARSPPEELATVRGLIVPIIKTTPVTLPFNLGQTVADNCLSLSGMGYHLGLGGYCPTCTASGEPRLCRTDRAALILAYVQQLNNIYEYRVFLASILALSDRANMQAASAEPLLSSVLAQPELFFMYHIMREGGMRDIRVLFYRDGDAGGFMMYVIFPGKSVHLHYRLIDHIQAACRGYKIVAHVWQTTFLLSVCRNPEQQTETVVPSIGTSDVYCKMCDLNFDGELLLEYKRLYALFDDFVPPR

SEQ ID NO: 6 - protein, 215 aa, Artificial Sequence
  VZV orf24 consisting of VZV orf24 (Uniprot entry: Q6QCN1, 16- GDNLLQRI .. TDAYM-189) is fused via a GGSGSGGS linker to VZV orf27 (Uniprot entry: Q6QCM8, 77-SKERSV.....RGLIVPII 99)
GDNLLQRIRLVVPSALQCCDGDLPIFDPQRPPARCVFQFNGEDNVSEAFPVEYIMRLMANWAQVDCDPYIKIQNTGVSVLFQGFFFRPTNAPVAEVSIDSNNVILSSTLSTGINLSALESIKRGGGIDRRPLQALMWVNCFVRMPYVQLSFRFMGPEDPSRTIKLMARATDAYMGGSGSGGSSKERSVYRHYFNYIARSPPEELATVRGLIVPII

SEQ ID NO: 7 - protein, 29 aa, Human cytomegalovirus
LTLHDLHDIFREHPELELKYLNMMKMAIT

SEQ ID NO: 8 - protein, 376 aa, Human cytomegalovirus
MSSVSGVRTPRERRSALRSLLRKRRQRELASKVASTVNGATSANNHGEPPSPADARPRLTLHDLHDIFREHPELELKYLNMMKMAITGKESICLPFNFHSHRQHTCLDISPYGNEQVSRIACTSCEDNRILPTASDAMVAFINQTSNIMKNRNFYYGFCKSSELLKLSTNQPPIFQIYYLLHAANHDIVPFMHAEDGRLHMHVIFENPDVHIPCDCITQMLTAAREDYSVTLNIVRDHVVISVLCHAVSASSVKIDVTILQRKIDEMDIPNDVSESFERYKELIQELCQSSGNNLYEEATSSYAIRSPLTASPLHVVSTNGCGPSSSSQSTPPHLHPPSQATQPHHYSHHQSQSQQHHHRPQSPPPPLFLNSIRAP

SEQ ID NO: 9 - protein, 397 aa, Human cytomegalovirus
MEMNKVLHQDLVQATRRILKLGPSELRVTDAGLICKNPNYSVCDAMLKTDTVYCVEYLLSYWESRTDHVPCFIFKNTGCAVSLCCFVRAPVKLVSPARHVGEFNVLKVNESLIVTLKDIEEIKPSAYGVLTKCVVRKSNSASVFNIELIAFGPENEGEYENLLRELYAKKAASTSLAVRNHVTVSSHSGSGPSLWRARMSAALTRTAGKRSSRTASPPPPPRHPSCSPTMVAAGGAAAGPRPPPPPMAAGSWRLCRCEACMGRCGCASEGDADEEEEELLALAGEGKAAAAAAGQDVGGSARRPLEEHVSRRRGVSTHHRHPPSPPCAPSLERTGYRWAPSSWWRARSGPSRPQSGPWLPARFATLGPLVLALLLVLALLWRGHGQSSSPTRSAHRD

SEQ ID NO: 10 - protein, 306 aa, human herpesvirus 1
MYDTDPHRRGSRPGPYHGKERRRSRSSAAGGTLGVVRRASRKSLPPHARKQELCLHERQRYRGLFAALAQTPSEEIAIVRSLSVPLVKTTPVSLPFCLDQTVADNCLTLSGMGYYLGIGGCCPACNAGDGRFAATSREALILAFVQQINTIFEHRAFLASLVVLADRHNAPLQDLLAGILGQPELFFVHTILRGGGACDPRLLFYPDPTYGGHMLYVIFPGTSAHLHYRLIDRMLTACPGYRFVAHVWQSTFVLVVRRNAEKPTDAEIPTVSAADIYCKMRDISFDGGLMLEYQRLYATFDEFPPP

SEQ ID NO: 11 - protein, 305 aa, human herpesvirus 2
MYDIAPRRSGSRPGPGRDKTRRRSRFSAAGNPGVERRASRKSLPSHARRLELCLHERRRYRGFFAALAQTPSEEIAIVRSLSVPLVKTTPVSLPFSLDQTVADNCLTLSGMGYYLGIGGCCPACSAGDGRLATVSREALILAFVQQINTIFEHRTFLASLVVLADRHSTPLQDLLADTLGQPELFFVHTILRGGGACDPRFLFYPDPTYGGHMLYVIFPGTSAHLHYRLIDRMLTACPGYRFAAHVWQSTFVLVVRRNAEKPADAEIPTVSAADIYCKMRDISFDGGLMLEYQRLYATFDEFPPP

SEQ ID NO: 12 - protein, 333 aa, Human herpesvirus 3
MHLKPTRFFHANQPPMPHSYEMEDLCFDDMQYRWSPSNTPYRSMSRRYKSVSRSGPSMRVRSRTPCRRQTIRGKLMSKERSVYRHYFNYIARSPPEELATVRGLIVPIIKTTPVTLPFNLGQTVADNCLSLSGMGYHLGLGGYCPTCTASGEPRLCRTDRAALILAYVQQLNNIYEYRVFLASILALSDRANMQAASAEPLLSSVLAQPELFFMYHIMREGGMRDIRVLFYRDGDAGGFMMYVIFPGKSVHLHYRLIDHIQAACRGYKIVAHVWQTTFLLSVCRNPEQQTETVVPSIGTSDVYCKMCDLNFDGELLLEYKRLYALFDDFVPPR

SEQ ID NO: 13 - protein, 264 aa, Human herpesvirus 6
MTVHKSRIRRSRSLSVTHRIQKRPDHREKTKLYLQLKLHDLHTVFNLFPEYEQKFLAIIKLPITGKEPIDVPFSLSNHHQHTCLEFSPYANEQISKSACLHCESVSVPTSSDAMVAHLNQVNNVMQNRLYFYGFRKDMELIRMSAKQPTIFQIFYIVHNTINNIFPIMFERKQKLGMHIVFQSRTLHIPCECIKQIVAVSSGYNVYLDILQESVILTVLCETLDTNTNIHIDIGMLQKKLEEMDIPNEISDRLEKYKGHLIGFH

SEQ ID NO: 14 - protein, 264 aa, Human herpesvirus 6B
MTVHKNRFRRSRSLSVTHRIQKRPDHREKTKLYLQLKLHDLHAVFNLFPEYEQKFLAIIKLPITGKEPIDVPFSLSNHHQHTCLEFSPYANEQISKSACLHCESVSVPTSSDAMVAHLNQVTNVMQNRFYFYGFRKDMELIRMSAKQPTIFQIFYIVHNTINNIFPIMFEKKQKLGMHIVFQSRTLHIPCECIKQIIAVSSGYNVYLDILQDSVILTVLCETLDTNTNIHIDIGMLQKKLEEMDIPNEISDRLEKYKGHLIGFH

SEQ ID NO: 15 - protein, 259 aa, Human herpesvirus 7
MAIQSTRRLRRASSLLKKSKPYNKEKTNLSLSLSLKELHSVFKLFPEYELKFLNMMKLPITGKEPIKIPFDLSLHHQHTCLDLSPYANEQVSKSACVNCGTTNIPTASDAMVAYMNQISNVMQNRLYYYGFQKKVELIRMSAKQPTLFQIFYILSSIASNFLPIMFENNEKLNMYVVFQTRTLHIPCECINQIMTVSSGYTVLLDILHDSIVLHVLCKTIETSNIQIDINVLQRKIEEMDVPDEIGDKFEKLKHILPFI

SEQ ID NO: 16 - protein, 318 aa, Human herpesvirus 4
MAPVTPDAVNARQQRPADPALRRLMHPHHRNYTASKASAHSVKSVSRCGKSRSELGRMERVGSVARSICSRHTRHGVDRSHFSLRDFFRGISANFELGKDFLREMNTPIHVSEAVFLPLSLCTLSPGRCLRLSPFGHSLTLGSHCEICINRSQVHVPQEFSSTQLSFFNNVHKIIPNKTFYVSLLSSSPSAVKAGLSQPSLLYAYLVTGHFCGTICPIFSTNGKGRLIMHLLLQGTSLHIPETCLKLLCENIGPTYELAVDLVGDAFCIKVSPRDTVYEKAVNVDEDAIYEAIKDLECGDELRLQIINYTQLILENKQ

SEQ ID NO: 17 - protein, 302 aa, Human herpesvirus 8
MPKSVSSHISLATSTGRSGPRDIRRCLSSRLRSVPPGARSASVSSKHRNGLRKFISDKVFFSILSHRHELGVDFLREMETPICTSKTVMLPLDLSTVAPGRCVSLSPFGHSSNMGFQCALCPSTENPTVAQGSRPQTMVGDALKKNNELCSVALAFYHHADKVIQHKTFYLSLLSHSMDVVRQSFLQPGLLYANLVLKTFGHDPLPIFTTNNGMLTMCILFKTRALHLGETALRLLMDNLPNYKISADCCRQSYVVKFVPTHPDTASIAVQVHTICEAVAALDCTDEMRDDIQKGTALVNAL

SEQ ID NO: 18 - protein, 271 aa, PrV
MFERRRLLRRKSSAARRKTLTRAARDRYAPYFAYAAAQPSDEVTTVRGLSNPLIKTAPVTLPFDLGQAVADNCLSLSGMGYYLGLGGCCPTCAAAEPRLGRSDRAALVLAYVQQLNSIYEYRVFLASVAARDPSERALEEVLAHPELFFAYYVLRDGGLRDVRVLFFEDPDAQGALMMYVVFPEKSVHVHHRVLDRLLGACAGHRIVAHVWQTMFVLVVRKKGDGRPADDVPAVSASDIYCKMRDISFDGELLLEYKRLYAAFEDFRPPRP

SEQ ID NO: 19 - protein, 333 aa, Mouse cytomegalovirus 1
MFRSPEGEERDAADREEEEGGEARRRSRMMMSPRRVKRARHRPAGSGLRTPLRSPSACRCSSPSPERQWQQRRRAEKRSTTPTDPPPPPKRSAASAAAGAAAPESEYLNVKLSELHDVFQRHPDLEQKYLKIMKLPITGKESIRLPFDFKSHRQHTCLDLSPYGNDQVSRSACTTCKETTRLPTASDSMVAFINQTSNVMKHRKFYFGFRKNMELLKMAANQPQLFQIYYIVQSCVQEIVPLIYYDREMAHMQLIFEKETVHIPSQCIEQILTVAKDAYGVSLDIAHQRITLTARCLRLESSSLRIDVLMLQRKVDELEIPNETNEKFESYSL

SEQ ID NO: 20 - protein, 275 aa, human herpesvirus 1
MAGLGKPYTGHPGDAFEGLVQRIRLIVPSTLRGGDGEAGPYSPSSLPSRCAFQFHGHDGSDESFPIEYVLRLMNDWAEVPCNPYLRIQNTGVSVLFQGFFHRPHNAPGGAITPERTNVILGSTETTGLSLGDLDTIKGRLGLDARPMMASMWISCFVRMPRVQLAFRFMGPEDAGRTRRILCRAAEQAITRRRRTRRSREAYGAEAGLGVAGTGFRARGDGFGPLPLLTQGPSRPWHQALRGLKHLRIGPPALVLAAGLVLGAAIWWVVGAGARL

SEQ ID NO: 21 - protein, 276 aa, human herpesvirus 2
MAGMGKPYGGRPGDAFEGLVQRIRLIVPATLRGGGGESGPYSPSNPPSRCAFQFHGQDGSDEAFPIEYVLRLMNDWADVPCNPYLRVQNTGVSVLFQGFFNRPHGAPGGAITAEQTNVILHSTETTGLSLGDLDDVKGRLGLDARPMMASMWISCFVRMPRVQLAFRFMGPEDAVRTRRILCRAAEQALARRRRSRRSQDDYGAVVVAAAHHSSGAPGPGVAASGPPAPPGRGPARPWHQAVQLFRAPRPGPPALLLLAAGLFLGAAIWWAVGARL

SEQ ID NO: 22 - protein, 269 aa, Human herpesvirus 3
MSRRTYVRSERRRGCGDNLLQRIRLVVPSALQCCDGDLPIFDPQRPPARCVFQFNGEDNVSEAFPVEYIMRLMANWAQVDCDPYIKIQNTGVSVLFQGFFFRPTNAPVAEVSIDSNNVILSSTLSTGINLSALESIKRGGGIDRRPLQALMWVNCFVRMPYVQLSFRFMGPEDPSRTIKLMARATDAYMYKETGNNLDEYIRWRPSFRSPPENGSPNTSVQMQSDIKPALPDTQTTRVWKLALPVANVTYALFIVIVLVVVLGAVLFWK

SEQ ID NO: 23 - protein, 276 aa, Human herpesvirus 6A
MANVLKEKMYDELLSATCRILKLGSHDYRITERNLLSKNPKFPLCDIILKLDYAYNLEYLLSLWEHVTKQEPRFVFKNTGGAVSMSCYLHAPVKVEGHHAVRECNILRVNECLTVRMSDIVAMKPSTFAVFTKCIIRRNRDDTYVVEFVAFGPENESEYISLLKAIFLKKCSMGKQHLESNRFCQGLRRRSSHVLEKGRFESSGKVVNKASAVVTSQESIKQFYEKEKSLLSGVKFWRLSERHCRFALVGICFLLALYFCYVLLKKTPTPASGSVV

SEQ ID NO: 24 - protein, 276 aa, Human herpesvirus 6B
MANVLKEKMYDELLSATCRILKLGSHDYRMTERNLLSKNPKFPLCDIILKLDYAYNLEYLLSLWEHVTKQEPRFVFKNTGGAVSMSCYLHAPVKAEGHHAVRECNILRVNECLTVRMSDIVAMKPSTFAVFTKCIIRRNRDETYVVEFVAFGPENESEYISLLKAIFLKKCSMGKQHLESNRFCQGLRRRSSHVLEKGQLGSSGEIANKASAVVTSQESINQFYEKEKSFLSGVKFSRLSERHCRVAIVSICFLLALYFCYVLLKKTPTPASGPVV

SEQ ID NO: 25 - protein, 258 aa, Human herpesvirus 7
MLKEKMYDELILSTCRVLKLGPADFRVTDKNLFSKNPKFPLCDILLKLDFAYSLEYLLSLWEDLTKQEARFIFKNTGGAVSMSCYLHAPIKQESQNIVKECNILNVNECLSVCLNDIEAIKPSSSGVLTKCIIRRNRDAAFIVEFVAFGPESESEYIALLKAIILKKKFLERQDLEKHRAARHIKKPLRLQLKSVGEMTSFRSINYMGNTKDAAVFPVTVPIFARRNNILCGFLVAALLIVCYVIFKEFALSADFSAV

SEQ ID NO: 26 - protein, 336 aa, Human herpesvirus 4
MASPEERLLDELNNVIVSFLCDSGSLEVERCSGAHVFSRGSSQPLCTVKLRHGQIYHLEFVYKFLAFKLKNCNYPSSPVFVISNNGLATTLRCFLHEPSGLRSGQSGPCLGLSTDVDLPKNSIIMLGQDDFIKFKSPLVFPAELDLLKSMVVCRAYITEHRTTMQFLVFQAANAQKASRVMDMISDMSQQLSRSGQVEDTGARVTGGGGPRPGVTHSGCLGDSHVRGRGGWDLDNFSEAETEDEASYAPWRDKDSWSESEAAPWKKELVRHPIRRHRTRETRRMRGSHSRVEHVPPETRETVVGGAWRYSWRATPYLARVLAVTAVALLLMFLRWT

SEQ ID NO: 27 - protein, 271 aa, Human herpesvirus 8
MSVVGKRVVDELCRVVSSYLGQSGQSLDLERCIDGAPVYAKGGATAICTVRMQHGCVYHLEFVYKFWAHLLEEMHYPFSPCFVISNNGLSTTLKCFLCRPSDAVSQFGHVLPVESDVYLAKNTSVVLGQDDFTKFKASLVFSKNLGVYNSMVICRTYFTDYRQVLQFLVVTPKSHKRLKSLLETVYCLAAPVADSAAQGGAGFPTNGRDARACTSDVTAVYWAGQGGRTVRILGAFQWSLGRAVALVRRSWPWISAGIAFLCLGLVWMRPS

SEQ ID NO: 28 - protein, 262 aa, PrV
MSGTLVQRLKLILSGGNLRCSDGETACDPERPPTRCVFQVHGQDGSNDTFPLEYVLRLMRSWAHVPCDPYVRVQNTGVSVLFQGFFFRPADAPLAAITAEHNNVILASTHSTGMSLSALDDIKRAGGVDTRPLRAMMSVSCFVRMPRVQLSFRFMGPDDASQTQRLLDRAEMRQRSVSRPGGGAGGGDDGEGPSPRAPIRPTVISPVPGHAAAAFVGQAAYPPPARFPASLLHTLLGLRRLAGYAVACVTGALAIVIILNMR

SEQ ID NO: 29 - protein, 316 aa, Mouse cytomegalovirus 1
MEIDKNVGADLISNTRRILRLDENELRITDTALICKNPNYSLCDAMLTTDIVYPVEYLLSYWECRSGRTACFVFKNTGCRVSLSCYIGFPERLKDLKRVCDFNFLSVNEALVVTLADIERIKPCDKGVLTNCVVRKSNSGMSYNIEVVAFGPDNEAEYQALLRDIYARRMTSVPTDCGSLICRRARCLAAAPPRRPPPPPPPGQRWGSLRKHGPVLTRRYAGGGGAAKNQPAAASPTSTSTSSPAAPSRDQDQTQRPPPAGDTNVTAAETTYSERTISFLTRHANAIHCALILAAAIALVLLWLLYWHAARSAGHP

SEQ ID NO: 30 - protein, 28 aa, human herpesvirus 1
RYRGLFAALAQTPSEEIAIVRSLSVPLV

SEQ ID NO: 31 - protein, 28 aa, human herpesvirus 2
RYRGFFAALAQTPSEEIAIVRSLSVPLV

SEQ ID NO: 32 - protein, 28 aa, Human herpesvirus 3
VYRHYFNYIARSPPEELATVRGLIVPII

SEQ ID NO: 33 - protein, 28 aa, Human herpesvirus 6A
KLHDLHTVFNLFPEYEQKFLAIIKLPIT

SEQ ID NO: 34 - protein, 28 aa, Human herpesvirus 6B
SLKELHSVFKLFPEYELKFLNMMKLPIT

SEQ ID NO: 35 - protein, 28 aa, Human herpesvirus 7
SLKELHSVFKLFPEYELKFLNMMKLPIT

SEQ ID NO: 36 - protein, 28 aa, Human herpesvirus 4
SLRDFFRGISANFELGKDFLREMNTPIH

SEQ ID NO: 37 - protein, 28 aa, Human herpesvirus 8
SDKVFFSILSHRHELGVDFLREMETPIC

SEQ ID NO: 38 - protein, 28 aa, PrV
RYAPYFAYAAAQPSDEVTTVRGLSNPLI

SEQ ID NO: 39 - protein, 28 aa, Mouse cytomegalovirus 1
KLSELHDVFQRHPDLEQKYLKIMKLPIT

SEQ ID NO: 40 - protein, 20 aa, Artificial Sequence
  Sequence for cloning purposes
MGSSHHHHHHSSGLVPRGSH

SEQ ID NO: 41 - protein, 8 aa, Artificial Sequence
  Flag peptide
DYKDDDDK

SEQ ID NO: 42 - DNA, 93 bp, Artificial Sequence
  Cloning sequence
taggaattcatgccgtcgccggccgacgcgcgcccgcgcctcacgctgcacgacctgcacgacatcttccgcgagcaccccgaactggagctc

SEQ ID NO: 43 - DNA, 57 bp, Artificial Sequence
  Restriction site for cloning
tagctcgagtcacttgtcgtcatcgtctttgtagtcgccgctggactgacacagctc

SEQ ID NO: 44 - DNA, 94 bp, Artificial Sequence
  5-BFLF2 (aa73) EcoRI
taggaattcatgaccagacatggtgtagacagatcccatttttcactacgggacttcttcaggggaatctctgccaactttgagctgggcaaag

SEQ ID NO: 45 - DNA, 58 bp, Artificial Sequence
  3-BFLF2 (aa318)-Flag XhoI
tagctcgagtcacttgtcgtcatcgtctttgtagtcctgtttattttccaaaatgagc

SEQ ID NO: 46 - DNA, 63 bp, Artificial Sequence
  5-UL53 globular(aa88) + BFLF2 Hook(aa95)
tttgagctgggcaaagattttctgcgtgagatgaacacccccatacatggcaaagagtccatc

SEQ ID NO: 47 - DNA, 94 bp, Artificial Sequence
  5-BFLF2 Hook(aa95) mit with UL53 Hook(aa50) EcoRI
taggaattcatgccgtcgccggccgacgcgcgcccgcgcctcacgctgcacgacctgcacgacatcttccgcgagcactttgagctgggcaaag

SEQ ID NO: 48 - DNA, 93 bp, Artificial Sequence
  5-UL53 Hook(aa72) with BFLF2 Hook(aa73) EcoRI
taggaattcatgaccagacatggtgtagacagatcccatttttcactacgggacttcttcaggggaatctctgccaaccccgaactggagctc

SEQ ID NO: 49 - DNA, 67 bp, Artificial Sequence
  5-BFLF2 globular(aa111) mit with UL53 Hook(aa72)
cccgaactggagctcaagtaccttaacatgatgaagatggccatcacggtctcagaggccgtgtttc

SEQ ID NO: 50 - DNA, 59 bp, Artificial Sequence
  5-BFRF1 EcoRI attB1
taggaattcggggacaagtttgtacaaaaaagcaggctaccatggcgagcccggaagag

SEQ ID NO: 51 - DNA, 31 bp, Artificial Sequence
  3-BFRF1-Linker BamHI
tagggatcccccggtccacctcagaaacatc

SEQ ID NO: 52 - DNA, 37 bp, Artificial Sequence
  5-BFLF2-Linker BamHI
tagggatccgggagcatggccccggtcaccccagatg

SEQ ID NO: 53 - DNA, 86 bp, Artificial Sequence
  3-BFLF2 XbaI attB2-Flag
tagtctagaggggaccactttgtacaagaaagctgggttcacttgtcgtcatcgtctttgtagtcctgtttattttccaaaatgag

SEQ ID NO: 54 - DNA, 49 bp, Artificial Sequence
  BGLF4 attB1
ggggacaagtttgtacaaaaaagcaggctaccatggatgtgaatatggc

SEQ ID NO: 55 - DNA, 74 bp, Artificial Sequence
  3-BGLF4 attB2-Flag
ggggaccactttgtacaagaaagctgggttcacttgtcgtcatcgtctttgtagtctccacgtcggccatctgg

SEQ ID NO: 56 - DNA, 21 bp, Artificial Sequence
  T7
ttaatacgactcactataggg

SEQ ID NO: 57 - DNA, 19 bp, Artificial Sequence
  SP6
catttaggtgacactatag

SEQ ID NO: 58 - DNA, 20 bp, Artificial Sequence
  5-pInd20seq_pCMV
ccatccacgctgttttgacc

SEQ ID NO: 59 - DNA, 18 bp, Artificial Sequence
  5-BFRF1-BFLF2 Seq.
actcgtggtcggaatccg

SEQ ID NO: 60 - DNA, 17 bp, Artificial Sequence
  3-pInducer20 Sequencing
ttactaagcgtagtctg

SEQ ID NO: 61 - protein, 14 aa, Human cytomegalovirus
  NLS (1)..(14): Residues 13 to 26 of HCMV pUL53
  HCMV-NLS (1)..(14): Residues 13 to 26 of HCMV pUL53
RRSALRSLLRKRRQ

SEQ ID NO: 62 - protein, 21 aa, Human cytomegalovirus
LHDLHDFREHPELELKYLNMM